European Patent Application EP 4 545 085 A1, published April 30, 2025. Title: CAR T-cells against CD79b for the treatment of Non-Hodgkin Lymphoma. Applicant: Fundacion Instituto de Investigacion Sanitaria de la Fundacion Jimenez Diaz. The sequence listing filed with the application follows.

SEQUENCE LISTING (32 sequences)

SEQ ID NO: 1 - protein, 12 aa, unidentified
KTSGYTFTDYWM

SEQ ID NO: 2 - protein, 17 aa, unidentified
MIDPSDSETHYNQMFKD

SEQ ID NO: 3 - protein, 4 aa, unidentified
NLNY

SEQ ID NO: 4 - protein, 113 aa, unidentified
QVQLQQPGAELVRPGASLKLSCKTSGYTFTDYWMNWVKQRPGQGLEWIGMIDPSDSETHYNQMFKDKATLTVDKSSSTAYMQLSSLTSEDSAVYYCTRNLNYWGQGTTLTVSS

SEQ ID NO: 5 - protein, 16 aa, unidentified
KSSQSLLDSDGKTYLN

SEQ ID NO: 6 - protein, 7 aa, unidentified
LVSKLAS

SEQ ID NO: 7 - protein, 9 aa, unidentified
WQGTHFPQT

SEQ ID NO: 8 - protein, 112 aa, unidentified
DVVLTQTPLSLSVTIGQPASISCKSSQSLLDSDGKTYLNWLLQRPGQSPERLIYLVSKLASGVPDRFTGSGSGTDFTLKINRVEAEDLGVYFCWQGTHFPQTFGAGTKLEIK

SEQ ID NO: 9 - protein, 240 aa, unidentified
QVQLQQPGAELVRPGASLKLSCKTSGYTFTDYWMNWVKQRPGQGLEWIGMIDPSDSETHYNQMFKDKATLTVDKSSSTAYMQLSSLTSEDSAVYYCTRNLNYWGQGTTLTVSSGGGGSGGGGSGGGGSDVVLTQTPLSLSVTIGQPASISCKSSQSLLDSDGKTYLNWLLQRPGQSPERLIYLVSKLASGVPDRFTGSGSGTDFTLKINRVEAEDLGVYFCWQGTHFPQTFGAGTKLEIK

SEQ ID NO: 10 - protein, 13 aa, unidentified
KASGYTFTTYWMN

SEQ ID NO: 11 - protein, 4 aa, unidentified
TLSY

SEQ ID NO: 12 - protein, 113 aa, unidentified
QVQLQQPGAELVRPGASVKLSCKASGYTFTTYWMNWVKQRPGQGLEWIGMIDPSDSETHYNQMFKDKATLTVDKSSTTAYMQLSSLTSEDSAVYYCARTLSYWGQGTLVTVSA

SEQ ID NO: 13 - protein, 7 aa, unidentified
LVSKLDS

SEQ ID NO: 14 - protein, 9 aa, unidentified
WQGTHFPLT

SEQ ID NO: 15 - protein, 112 aa, unidentified
DVVMTQTPLTLSVTIGQPASISCKSSQSLLDSDGKTYLNWLLQRPGQSPKPLISLVSKLDSGVPVRFTGSGSGTDFTLKISRVEAEDLGVYYCWQGTHFPLTFGGGTKLEIK

SEQ ID NO: 16 - protein, 240 aa, unidentified
QVQLQQPGAELVRPGASVKLSCKASGYTFTTYWMNWVKQRPGQGLEWIGMIDPSDSETHYNQMFKDKATLTVDKSSTTAYMQLSSLTSEDSAVYYCARTLSYWGQGTLVTVSAGGGGSGGGGSGGGGSDVVMTQTPLTLSVTIGQPASISCKSSQSLLDSDGKTYLNWLLQRPGQSPKPLISLVSKLDSGVPVRFTGSGSGTDFTLKISRVEAEDLGVYYCWQGTHFPLTFGGGTKLEIK

SEQ ID NO: 17 - protein, 13 aa, unidentified
KASGYTFTSYWMN

SEQ ID NO: 18 - protein, 17 aa, unidentified
MIDPSDSETHYNQMFRD

SEQ ID NO: 19 - protein, 4 aa, unidentified
ALGY

SEQ ID NO: 20 - protein, 113 aa, unidentified
QVQLQQPGAELVRPGASVKLSCKASGYTFTSYWMNWVKQRPGQGLEWIGMIDPSDSETHYNQMFRDKATLTVDKPSNTAYMQLSRLTSEDSAVYYCARALGYWGQGTSVTVSS

SEQ ID NO: 21 - protein, 112 aa, unidentified
DVVMTQTPLTLSVTIGQPASISCKSSQSLLDSDGKTYLNWLLQRPGQSPNRLIYLVSKLDSGVPDRFTGSGSGTDFTLKISRVEAEDLGVYYCWQGTHFPLTFGGGTKLELK

SEQ ID NO: 22 - protein, 240 aa, unidentified
QVQLQQPGAELVRPGASVKLSCKASGYTFTSYWMNWVKQRPGQGLEWIGMIDPSDSETHYNQMFRDKATLTVDKPSNTAYMQLSRLTSEDSAVYYCARALGYWGQGTSVTVSSGGGGSGGGGSGGGGSDVVMTQTPLTLSVTIGQPASISCKSSQSLLDSDGKTYLNWLLQRPGQSPNRLIYLVSKLDSGVPDRFTGSGSGTDFTLKISRVEAEDLGVYYCWQGTHFPLTFGGGTKLELK

SEQ ID NO: 23 - protein, 20 aa, unidentified
MEAPAQLLFLLLLWLPDTTG

SEQ ID NO: 24 - protein, 15 aa, unidentified
GGGGSGGGGSGGGGS

SEQ ID NO: 25 - protein, 46 aa, unidentified
TTTPAPRPPTPAPTIASQPLSLRPEACRPAAGGAVHTRGLDFACDI

SEQ ID NO: 26 - protein, 23 aa, unidentified
YIWAPLAGTCGVLLLSLVITLYC

SEQ ID NO: 27 - protein, 69 aa, unidentified
TTTPAPRPPTPAPTIASQPLSLRPEACRPAAGGAVHTRGLDFACDIYIWAPLAGTCGVLLLSLVITLYC

SEQ ID NO: 28 - protein, 42 aa, unidentified
KRGRKKLLYIFKQPFMRPVQTTQEEDGCSCRFPEEEEGGCEL

SEQ ID NO: 29 - protein, 113 aa, unidentified
RVKFSRSADAPAYQQGQNQLYNELNLGRREEYDVLDKRRGRDPEMGGKPQRRKNPQEGLYNELQKDKMAEAYSEIGMKGERRRGKGHDGLYQGLSTATKDTYDALHMQALPPR

SEQ ID NO: 30 - DNA, 720 bp, unidentified
  source 1..720: mol_type = other DNA
caggtccagcttcagcagccgggtgctgaattggtaagacctggcgcgtctcttaaactgagttgtaaaacgtctggatataccttcaccgactactggatgaactgggttaaacaaagaccgggacagggtttggaatggattggtatgatagatcctagtgattcagaaactcactataatcaaatgttcaaagacaaagctacactcaccgttgacaaatcttcttctacggcttatatgcagctcagctccctcaccagcgaggacagtgccgtttattactgcactcgcaacttgaattactggggacagggaacgactttgaccgtcagtagcggcggcgggggatcaggcggcggtggttctggcgggggtggctccgatgtggttttgactcaaacaccactttcacttagtgttactattggtcaaccggccagcatatcttgtaagtctagccaaagtttgctggattccgacgggaaaacatacttgaactggctgctccaacgcccaggacagtcccctgaaagattgatatacctcgtatctaaactggcaagcggagtgccagatcgctttaccgggagcggatctggtactgatttcactctgaaaatcaatagagttgaagccgaggacctcggcgtatatttttgctggcagggtacccactttccgcaaacatttggcgctgggacgaagctggaaattaaa

SEQ ID NO: 31 - DNA, 720 bp, unidentified
  source 1..720: mol_type = other DNA
caagtgcaactgcagcagcccggggcggaactggttcggcccggggcgagtgtgaaacttagctgcaaagcttccggatacacattcactacgtactggatgaactgggttaaacaaaggcctgggcagggcctcgagtggatcgggatgatagacccgtctgattctgaaacccattataaccaaatgttcaaagacaaggcgacgttgacagtagataagtcttctacgactgcctacatgcaattgagcagtttgacaagtgaagattcagctgtgtattactgtgcgagaaccctgtcatactggggccaaggtactctcgtaaccgttagtgccggaggaggcggctctggaggaggtggatccggtggtggtggttcagacgtagttatgacacaaactcctttgacactcagcgtaacgatcggacagccggcttcaattagttgcaaaagtagtcagtctttgctcgactcagatggcaagacgtatctgaactggcttctgcagcgccccggacagagccctaaaccactgatatccctggtctctaagcttgatagtggcgttcctgtgcgcttcacggggagcggtagcggaaccgatttcacacttaagatttctagagtggaagcagaggacttgggcgtatattattgctggcaggggacacacttccctctgactttcggaggcggaactaaactcgaaataaaa

SEQ ID NO: 32 - DNA, 720 bp, unidentified
  source 1..720: mol_type = other DNA
caggttcaactgcaacaaccaggagcggagctggtccgaccgggggctagtgtcaaattgtcatgtaaggcaagtggatatacttttacaagctattggatgaattgggtaaagcagcgacccgggcaagggcttgagtggattggcatgattgaccctagtgactcagagacccactacaaccagatgttcagagacaaggcaaccttgacagttgacaagccaagtaatactgcgtatatgcagttgagtcgacttacatcagaggactctgcagtgtattattgcgctagggcactcggctattggggacaagggacctccgtcaccgtatcttccggaggtggtggatctggaggaggcggatctggtggcggggggtccgacgtcgttatgacccagactccacttacactctccgttacgattggacagcccgcttcaataagttgtaaaagttcccagtcactgctcgacagcgatggtaagacgtacctcaactggttgctccaaagacccggccaaagccccaaccgcctgatctatctcgtcagtaaattggattccggtgtccctgacaggttcacgggttctggtagcgggacagactttacgctcaaaatatctagagttgaagcagaagatcttggagtttattattgttggcaagggacgcactttccgcttacgttcgggggagggactaaacttgaactcaaa